European Patent Application EP 4 647 503 A1, published November 12, 2025. Title: ヒト細胞におけるインスリン分泌能の定量方法. Applicant: 学校法人順天堂. Application JP, filed January 4, 2024. The sequence listing filed with the application follows.

SEQUENCE LISTING (72 sequences)

SEQ ID NO: 1 - protein, 11 aa, synthetic construct
  source 1..11: note = HiBit
VSGWRLFKKIS

SEQ ID NO: 2 - protein, 31 aa, Homo sapiens
  source 1..31: note = C-peptide sequence
EAEDLQVGQVELGGGPGAGSLQPLALEGSLQ

SEQ ID NO: 3 - protein, 35 aa, synthetic construct
  source 1..35: note = C-peptide-like sequence
RREAEDLQVGQVELGGGPGAGSLQPLALEGSLQKR

SEQ ID NO: 4 - protein, 30 aa, synthetic construct
  source 1..30: note = C-peptide-like sequence
RREAEDLQVGGGPGAGSLQPLALEGSLQKR

SEQ ID NO: 5 - protein, 26 aa, synthetic construct
  source 1..26: note = C-peptide-like sequence
EAEDLQVGGGPGAGSLQPLALEGSLQ

SEQ ID NO: 6 - protein, 33 aa, synthetic construct
  source 1..33: note = C-peptide-like sequence
RREAEDLQVGQVELGGGPGAGSLQPLALEGSLQ

SEQ ID NO: 7 - protein, 33 aa, synthetic construct
  source 1..33: note = C-peptide-like sequence
EAEDLQVGQVELGGGPGAGSLQPLALEGSLQKR

SEQ ID NO: 8 - DNA, 5224 bp, synthetic construct
  source 1..5224: mol_type = other DNA; note = mIns1-Hibit1 expression plasmid
caactttgtatagaaaagttgctcgacattgattattgactagttattaatagtaatcaattacggggtcattagttcatagcccatatatggagttccgcgttacataacttacggtaaatggcccgcctggctgaccgcccaacgacccccgcccattgacgtcaataatgacgtatgttcccatagtaacgccaatagggactttccattgacgtcaatgggtggagtatttacggtaaactgcccacttggcagtacatcaagtgtatcatatgccaagtacgccccctattgacgtcaatgacggtaaatggcccgcctggcattatgcccagtacatgaccttatgggactttcctacttggcagtacatctacgtattagtcatcgctattaccatggtcgaggtgagccccacgttctgcttcactctccccatctcccccccctccccacccccaattttgtatttatttattttttaattattttgtgcagcgatgggggcggggggggggggggggcgcgcgccaggcggggcggggcggggcgaggggcggggcggggcgaggcggagaggtgcggcggcagccaatcagagcggcgcgctccgaaagtttccttttatggcgaggcggcggcggcggcggccctataaaaagcgaagcgcgcggcgggcgggagtcgctgcgcgctgccttcgccccgtgccccgctccgccgccgcctcgcgccgcccgccccggctctgactgaccgcgttactcccacaggtgagcgggcgggacggcccttctcctccgggctgtaattagcgcttggtttaatgacggcttgtttcttttctgtggctgcgtgaaagccttgaggggctccgggagggccctttgtgcggggggagcggctcggggggtgcgtgcgtgtgtgtgtgcgtggggagcgccgcgtgcggctccgcgctgcccggcggctgtgagcgctgcgggcgcggcgcggggctttgtgcgctccgcagtgtgcgcgaggggagcgcggccgggggcggtgccccgcggtgcggggggggctgcgaggggaacaaaggctgcgtgcggggtgtgtgcgtgggggggtgagcagggggtgtgggcgcgtcggtcgggctgcaaccccccctgcacccccctccccgagttgctgagcacggcccggcttcgggtgcggggctccgtacggggcgtggcgcggggctcgccgtgccgggcggggggtggcggcaggtgggggtgccgggcggggcggggccgcctcgggccggggagggctcgggggaggggcgcggcggcccccggagcgccggcggctgtcgaggcgcggcgagccgcagccattgccttttatggtaatcgtgcgagagggcgcagggacttcctttgtcccaaatctgtgcggagccgaaatctgggaggcgccgccgcaccccctctagcgggcgcggggcgaagcggtgcggcgccggcaggaaggaaatgggcggggagggccttcgtgcgtcgccgcgccgccgtccccttctccctctccagcctcggggctgtccgcggggggacggctgccttcgggggggacggggcagggcggggttcggcttctggcgtgtgaccggcggctctagagcctctgctaaccatgttcatgccttcttctttttcctacagctcctgggcaacgtgctggttattgtgctgtctcatcattttggcaaagaattgcaagtttgtacaaaaaagcaggctgccaccatggccctgttggtgcacttcctacccctgctggccctgcttgccctctgggagcccaaacccacccaggcttttgtcaaacagcatctttgtggtccccacctggtagaggctctctacctggtgtgtggggagcgtggcttcttctacacacccaagtcccgccgtgaagtggaggacccacaagtggaacaactggagctgggagtgagcggctggcggctgttcaagaagattagcggaagccccggggaccttcagaccttggcgttggaggtggcccggcagaagcgtggcattgtggatcagtgctgcaccagcatctgctccctctaccagctggagaactactgcaacggaagcggagccacgaacttctctctgttaaagcaagcaggagatgttgaagaaaaccccgggcctatggtgagcaagggcgaggagctgttcaccggggtggtgcccatcctggtcgagctggacggcgacgtaaacggccacaagttcagcgtgtccggcgagggcgagggcgatgccacctacggcaagctgaccctgaagttcatctgcaccaccggcaagctgcccgtgccctggcccaccctcgtgaccaccctgacctacggcgtgcagtgcttcagccgctaccccgaccacatgaagcagcacgacttcttcaagtccgccatgcccgaaggctacgtccaggagcgcaccatcttcttcaaggacgacggcaactacaagacccgcgccgaggtgaagttcgagggcgacaccctggtgaaccgcatcgagctgaagggcatcgacttcaaggaggacggcaacatcctggggcacaagctggagtacaactacaacagccacaacgtctatatcatggccgacaagcagaagaacggcatcaaggtgaacttcaagatccgccacaacatcgaggacggcagcgtgcagctcgccgaccactaccagcagaacacccccatcggcgacggccccgtgctgctgcccgacaaccactacctgagcacccagtccgccctgagcaaagaccccaacgagaagcgcgatcacatggtcctgctggagttcgtgaccgccgccgggatcactctcggcatggacgagctgtacaagtaaacccagctttcttgtacaaagtggtgatggccggccgcttcgagcagacatgataagatacattgatgagtttggacaaaccacaactagaatgcagtgaaaaaaatgctttatttgtgaaatttgtgatgctattgctttatttgtaaccattataagctgcaataaacaagttaacaacaacaattgcattcattttatgtttcaggttcagggggaggtgtgggaggttttttaaagcaagtaaaacctctacaaatgtggtagcggccgcggcgctcttccgcttcctcgctcactgactcgctgcgctcggtcgttcggctgcggcgagcggtatcagctcactcaaaggcggtaatacggttatccacagaatcaggggataacgcaggaaagaacatgtgagcaaaaggccagcaaaaggccaggaaccgtaaaaaggccgcgttgctggcgtttttccataggctccgcccccctgacgagcatcacaaaaatcgacgctcaagtcagaggtggcgaaacccgacaggactataaagataccaggcgtttccccctggaagctccctcgtgcgctctcctgttccgaccctgccgcttaccggatacctgtccgcctttctctcttcgggaagcgtggcgctttctcatagctcacgctgtaggtatctcagttcggtgtaggtcgttcgctccaagctgggctgtgtgcacgaaccccccgttcagcccgaccgctgcgccttatccggtaactatcgtcttgagtccaacccggtaagacacgacttatcgccactggcagcagccactggtaacaggattagcagagcgaggtatgtaggcggtgctacagagttcttgaagtggtggcctaactacggctacactagaagaacagtatttggtatctgcgctctgctgaagccagttaccttcggaaaaagagttggtagctcttgatccggcaaacaaaccaccgctggtagcggtggtttttttgtttgcaagcagcagattacgcgcagaaaaaaaggatctcaagaagatcctttgatcttttctacggggtctgacgctcagtggaacgaaaactcacgttaagggattttggtcatgagattatcaaaaaggatcttcacctagatccttttaaattaaaaatgaagttttaaatcaatctaaagtatatatgagtaaacttggtctgacagttaccaatgcttaatcagtgaggcacctatctcagcgatctgtctatttcgttcatccatagttgcctgactccccgtcgtgtagataactacgatacgggagggcttaccatctggccccagtgctgcaatgataccgcgagacccacgctcaccggctccagatttatcagcaataaaccagccagccggaagggccgagcgcagaagtggtcctgcaactttatccgcctccatccagtctattaattgttgccgggaagctagagtaagtagttcgccagttaatagtttgcgcaacgttgttgccattgctacaggcatcgtggtgtcacgctcgtcgtttggtatggcttcattcagctccggttcccaacgatcaaggcgagttacatgatcccccatgttgtgcaaaaaagcggttagctccttcggtcctccgatcgttgtcagaagtaagttggccgcagtgttatcactcatggttatggcagcactgcataattctcttactgtcatgccatccgtaagatgcttttctgtgactggtgagtactcaaccaagtcattctgagaatagtgtatgcggcgaccgagttgctcttgcccggcgtcaatacgggataataccgcgccacatagcagaactttaaaagtgctcatcattggaaaacgttcttcggggcgaaaactctcaaggatcttaccgctgttgagatccagttcgatgtaacccactcgtgcacccaactgatcttcagcatcttttactttcaccagcgtttctgggtgagcaaaaacaggaaggcaaaatgccgcaaaaaagggaataagggcgacacggaaatgttgaatactcatactcttcctttttcaatattattgaagcatttatcagggttattgtctcatgagcggatacatatttgaatgtatttagaaaaataaacaaataggggttccgcgcacatttccccgaaaagtgccacctgacgtctaagaaaccattattatcatgacattaacctataaaaataggcgtatcacgaggccctttcgtcggcgcgccgcggccgc

SEQ ID NO: 9 - DNA, 357 bp, synthetic construct
  source 1..357: mol_type = other DNA; note = mIns1-Hibit1 coding gene
atggccctgttggtgcacttcctacccctgctggccctgcttgccctctgggagcccaaacccacccaggcttttgtcaaacagcatctttgtggtccccacctggtagaggctctctacctggtgtgtggggagcgtggcttcttctacacacccaagtcccgccgtgaagtggaggacccacaagtggaacaactggagctgggagtgagcggctggcggctgttcaagaagattagcggaagccccggggaccttcagaccttggcgttggaggtggcccggcagaagcgtggcattgtggatcagtgctgcaccagcatctgctccctctaccagctggagaactactgcaac

SEQ ID NO: 10 - protein, 119 aa, synthetic construct
  source 1..119: note = mIns1-Hibit1
MALLVHFLPLLALLALWEPKPTQAFVKQHLCGPHLVEALYLVCGERGFFYTPKSRREVEDPQVEQLELGVSGWRLFKKISGSPGDLQTLALEVARQKRGIVDQCCTSICSLYQLENYCN

SEQ ID NO: 11 - DNA, 333 bp, synthetic construct
  source 1..333: mol_type = other DNA; note = mIns1-Hibit2 coding gene
atggccctgttggtgcacttcctacccctgctggccctgcttgccctctgggagcccaaacccacccaggcttttgtcaaacagcatctttgtggtccccacctggtagaggctctctacctggtgtgtggggagcgtggcttcttctacacacccaagtcccgccgtgaagtggaggacccacaagtggaacaactggagctgggaggagtgagcggctggcggctgttcaagaagattagcgcgttggaggtggcccggcagaagcgtggcattgtggatcagtgctgcaccagcatctgctccctctaccagctggagaactactgcaac

SEQ ID NO: 12 - protein, 111 aa, synthetic construct
  source 1..111: note = mIns1-Hibit2
MALLVHFLPLLALLALWEPKPTQAFVKQHLCGPHLVEALYLVCGERGFFYTPKSRREVEDPQVEQLELGGVSGWRLFKKISALEVARQKRGIVDQCCTSICSLYQLENYCN

SEQ ID NO: 13 - DNA, 336 bp, synthetic construct
  source 1..336: mol_type = other DNA; note = mIns1-Hibit3 coding gene
atggccctgttggtgcacttcctacccctgctggccctgcttgccctctgggagcccaaacccacccaggcttttgtcaaacagcatctttgtggtccccacctggtagaggctctctacctggtgtgtggggagcgtggcttcttctacacacccaagtcccgccgtgaagtggaggacccagtgagcggctggcggctgttcaagaagattagcggaggaagccccggggaccttcagaccttggcgttggaggtggcccggcagaagcgtggcattgtggatcagtgctgcaccagcatctgctccctctaccagctggagaactactgcaac

SEQ ID NO: 14 - protein, 112 aa, synthetic construct
  source 1..112: note = mIns1-Hibit3
MALLVHFLPLLALLALWEPKPTQAFVKQHLCGPHLVEALYLVCGERGFFYTPKSRREVEDPVSGWRLFKKISGGSPGDLQTLALEVARQKRGIVDQCCTSICSLYQLENYCN

SEQ ID NO: 15 - DNA, 342 bp, synthetic construct
  source 1..342: mol_type = other DNA; note = mIns1-Hibit4 coding gene
atggccctgttggtgcacttcctacccctgctggccctgcttgccctctgggagcccaaacccacccaggcttttgtcaaacagcatctttgtggtccccacctggtagaggctctctacctggtgtgtggggagcgtggcttcttctacacacccaagtcccgccgtgaagtggaggacccacaagtggaacaactggagctgggaggaagcgtgagcggctggcggctgttcaagaagattagcaccttggcgttggaggtggcccggcagaagcgtggcattgtggatcagtgctgcaccagcatctgctccctctaccagctggagaactactgcaac

SEQ ID NO: 16 - protein, 114 aa, synthetic construct
  source 1..114: note = mIns1-Hibit4
MALLVHFLPLLALLALWEPKPTQAFVKQHLCGPHLVEALYLVCGERGFFYTPKSRREVEDPQVEQLELGGSVSGWRLFKKISTLALEVARQKRGIVDQCCTSICSLYQLENYCN

SEQ ID NO: 17 - DNA, 342 bp, synthetic construct
  source 1..342: mol_type = other DNA; note = mIns1-Hibit5 coding gene
atggccctgttggtgcacttcctacccctgctggccctgcttgccctctgggagcccaaacccacccaggcttttgtcaaacagcatctttgtggtccccacctggtagaggctctctacctggtgtgtggggagcgtggcttcttctacacacccaagtcccgccgtgaagtggaggacccacaagtggtgagcggctggcggctgttcaagaagattagcggaggaagccccggggaccttcagaccttggcgttggaggtggcccggcagaagcgtggcattgtggatcagtgctgcaccagcatctgctccctctaccagctggagaactactgcaac

SEQ ID NO: 18 - protein, 114 aa, synthetic construct
  source 1..114: note = mIns1-Hibit5
MALLVHFLPLLALLALWEPKPTQAFVKQHLCGPHLVEALYLVCGERGFFYTPKSRREVEDPQVVSGWRLFKKISGGSPGDLQTLALEVARQKRGIVDQCCTSICSLYQLENYCN

SEQ ID NO: 19 - DNA, 5221 bp, synthetic construct
  source 1..5221: mol_type = other DNA; note = mIns2-Hibit1 expression plasmid
caactttgtatagaaaagttgctcgacattgattattgactagttattaatagtaatcaattacggggtcattagttcatagcccatatatggagttccgcgttacataacttacggtaaatggcccgcctggctgaccgcccaacgacccccgcccattgacgtcaataatgacgtatgttcccatagtaacgccaatagggactttccattgacgtcaatgggtggagtatttacggtaaactgcccacttggcagtacatcaagtgtatcatatgccaagtacgccccctattgacgtcaatgacggtaaatggcccgcctggcattatgcccagtacatgaccttatgggactttcctacttggcagtacatctacgtattagtcatcgctattaccatggtcgaggtgagccccacgttctgcttcactctccccatctcccccccctccccacccccaattttgtatttatttattttttaattattttgtgcagcgatgggggcggggggggggggggggcgcgcgccaggcggggcggggcggggcgaggggcggggcggggcgaggcggagaggtgcggcggcagccaatcagagcggcgcgctccgaaagtttccttttatggcgaggcggcggcggcggcggccctataaaaagcgaagcgcgcggcgggcgggagtcgctgcgcgctgccttcgccccgtgccccgctccgccgccgcctcgcgccgcccgccccggctctgactgaccgcgttactcccacaggtgagcgggcgggacggcccttctcctccgggctgtaattagcgcttggtttaatgacggcttgtttcttttctgtggctgcgtgaaagccttgaggggctccgggagggccctttgtgcggggggagcggctcggggggtgcgtgcgtgtgtgtgtgcgtggggagcgccgcgtgcggctccgcgctgcccggcggctgtgagcgctgcgggcgcggcgcggggctttgtgcgctccgcagtgtgcgcgaggggagcgcggccgggggcggtgccccgcggtgcggggggggctgcgaggggaacaaaggctgcgtgcggggtgtgtgcgtgggggggtgagcagggggtgtgggcgcgtcggtcgggctgcaaccccccctgcacccccctccccgagttgctgagcacggcccggcttcgggtgcggggctccgtacggggcgtggcgcggggctcgccgtgccgggcggggggtggcggcaggtgggggtgccgggcggggcggggccgcctcgggccggggagggctcgggggaggggcgcggcggcccccggagcgccggcggctgtcgaggcgcggcgagccgcagccattgccttttatggtaatcgtgcgagagggcgcagggacttcctttgtcccaaatctgtgcggagccgaaatctgggaggcgccgccgcaccccctctagcgggcgcggggcgaagcggtgcggcgccggcaggaaggaaatgggcggggagggccttcgtgcgtcgccgcgccgccgtccccttctccctctccagcctcggggctgtccgcggggggacggctgccttcgggggggacggggcagggcggggttcggcttctggcgtgtgaccggcggctctagagcctctgctaaccatgttcatgccttcttctttttcctacagctcctgggcaacgtgctggttattgtgctgtctcatcattttggcaaagaattgcaagtttgtacaaaaaagcaggctgccaccatggccctgtggatgcgcttcctgcccctgctggccctgctcttcctctgggagtcccaccccacccaggcttttgtcaagcagcacctttgtggttcccacctggtggaggctctctacctggtgtgtggggagcgtggcttcttctacacacccatgtcccgccgtgaagtggaggacccacaagtggcacaactggagctgggtgtgagcggctggcggctgttcaagaagattagcggaggcccgggagcaggtgaccttcagaccttggcactggaggtggcccagcagaagcgtggcattgtagatcagtgctgcaccagcatctgctccctctaccagctggagaactactgcaacggaagcggagccacgaacttctctctgttaaagcaagcaggagatgttgaagaaaaccccgggcctatggtgagcaagggcgaggaggataacatggccatcatcaaggagttcatgcgcttcaaggtgcacatggagggctccgtgaacggccacgagttcgagatcgagggcgagggcgagggccgcccctacgagggcacccagaccgccaagctgaaggtgaccaagggtggccccctgcccttcgcctgggacatcctgtcccctcagttcatgtacggctccaaggcctacgtgaagcaccccgccgacatccccgactacttgaagctgtccttccccgagggcttcaagtgggagcgcgtgatgaacttcgaggacggcggcgtggtgaccgtgacccaggactcctccctgcaggacggcgagttcatctacaaggtgaagctgcgcggcaccaacttcccctccgacggccccgtaatgcagaagaagaccatgggctgggaggcctcctccgagcggatgtaccccgaggacggcgccctgaagggcgagatcaagcagaggctgaagctgaaggacggcggccactacgacgctgaggtcaagaccacctacaaggccaagaagcccgtgcagctgcccggcgcctacaacgtcaacatcaagttggacatcacctcccacaacgaggactacaccatcgtggaacagtacgaacgcgccgagggccgccactccaccggcggcatggacgagctgtacaagtaaacccagctttcttgtacaaagtggtgatggccggccgcttcgagcagacatgataagatacattgatgagtttggacaaaccacaactagaatgcagtgaaaaaaatgctttatttgtgaaatttgtgatgctattgctttatttgtaaccattataagctgcaataaacaagttaacaacaacaattgcattcattttatgtttcaggttcagggggaggtgtgggaggttttttaaagcaagtaaaacctctacaaatgtggtagcggccgcggcgctcttccgcttcctcgctcactgactcgctgcgctcggtcgttcggctgcggcgagcggtatcagctcactcaaaggcggtaatacggttatccacagaatcaggggataacgcaggaaagaacatgtgagcaaaaggccagcaaaaggccaggaaccgtaaaaaggccgcgttgctggcgtttttccataggctccgcccccctgacgagcatcacaaaaatcgacgctcaagtcagaggtggcgaaacccgacaggactataaagataccaggcgtttccccctggaagctccctcgtgcgctctcctgttccgaccctgccgcttaccggatacctgtccgcctttctctcttcgggaagcgtggcgctttctcatagctcacgctgtaggtatctcagttcggtgtaggtcgttcgctccaagctgggctgtgtgcacgaaccccccgttcagcccgaccgctgcgccttatccggtaactatcgtcttgagtccaacccggtaagacacgacttatcgccactggcagcagccactggtaacaggattagcagagcgaggtatgtaggcggtgctacagagttcttgaagtggtggcctaactacggctacactagaagaacagtatttggtatctgcgctctgctgaagccagttaccttcggaaaaagagttggtagctcttgatccggcaaacaaaccaccgctggtagcggtggtttttttgtttgcaagcagcagattacgcgcagaaaaaaaggatctcaagaagatcctttgatcttttctacggggtctgacgctcagtggaacgaaaactcacgttaagggattttggtcatgagattatcaaaaaggatcttcacctagatccttttaaattaaaaatgaagttttaaatcaatctaaagtatatatgagtaaacttggtctgacagttaccaatgcttaatcagtgaggcacctatctcagcgatctgtctatttcgttcatccatagttgcctgactccccgtcgtgtagataactacgatacgggagggcttaccatctggccccagtgctgcaatgataccgcgagacccacgctcaccggctccagatttatcagcaataaaccagccagccggaagggccgagcgcagaagtggtcctgcaactttatccgcctccatccagtctattaattgttgccgggaagctagagtaagtagttcgccagttaatagtttgcgcaacgttgttgccattgctacaggcatcgtggtgtcacgctcgtcgtttggtatggcttcattcagctccggttcccaacgatcaaggcgagttacatgatcccccatgttgtgcaaaaaagcggttagctccttcggtcctccgatcgttgtcagaagtaagttggccgcagtgttatcactcatggttatggcagcactgcataattctcttactgtcatgccatccgtaagatgcttttctgtgactggtgagtactcaaccaagtcattctgagaatagtgtatgcggcgaccgagttgctcttgcccggcgtcaatacgggataataccgcgccacatagcagaactttaaaagtgctcatcattggaaaacgttcttcggggcgaaaactctcaaggatcttaccgctgttgagatccagttcgatgtaacccactcgtgcacccaactgatcttcagcatcttttactttcaccagcgtttctgggtgagcaaaaacaggaaggcaaaatgccgcaaaaaagggaataagggcgacacggaaatgttgaatactcatactcttcctttttcaatattattgaagcatttatcagggttattgtctcatgagcggatacatatttgaatgtatttagaaaaataaacaaataggggttccgcgcacatttccccgaaaagtgccacctgacgtctaagaaaccattattatcatgacattaacctataaaaataggcgtatcacgaggccctttcgtcggcgcgccgcggccgc

SEQ ID NO: 20 - DNA, 363 bp, synthetic construct
  source 1..363: mol_type = other DNA; note = mIns2-Hibit1 coding gene
atggccctgtggatgcgcttcctgcccctgctggccctgctcttcctctgggagtcccaccccacccaggcttttgtcaagcagcacctttgtggttcccacctggtggaggctctctacctggtgtgtggggagcgtggcttcttctacacacccatgtcccgccgtgaagtggaggacccacaagtggcacaactggagctgggtgtgagcggctggcggctgttcaagaagattagcggaggcccgggagcaggtgaccttcagaccttggcactggaggtggcccagcagaagcgtggcattgtagatcagtgctgcaccagcatctgctccctctaccagctggagaactactgcaac

SEQ ID NO: 21 - protein, 121 aa, synthetic construct
  source 1..121: note = mIns2-Hibit1
MALWMRFLPLLALLFLWESHPTQAFVKQHLCGSHLVEALYLVCGERGFFYTPMSRREVEDPQVAQLELGVSGWRLFKKISGGPGAGDLQTLALEVAQQKRGIVDQCCTSICSLYQLENYCN

SEQ ID NO: 22 - DNA, 339 bp, synthetic construct
  source 1..339: mol_type = other DNA; note = mIns2-Hibit2 coding gene
atggccctgtggatgcgcttcctgcccctgctggccctgctcttcctctgggagtcccaccccacccaggcttttgtcaagcagcacctttgtggttcccacctggtggaggctctctacctggtgtgtggggagcgtggcttcttctacacacccatgtcccgccgtgaagtggaggacccacaagtggcacaactggagctgggtggaggcgtgagcggctggcggctgttcaagaagattagcttggcactggaggtggcccagcagaagcgtggcattgtagatcagtgctgcaccagcatctgctccctctaccagctggagaactactgcaac

SEQ ID NO: 23 - protein, 113 aa, synthetic construct
  source 1..113: note = mIns2-Hibit2
MALWMRFLPLLALLFLWESHPTQAFVKQHLCGSHLVEALYLVCGERGFFYTPMSRREVEDPQVAQLELGGGVSGWRLFKKISLALEVAQQKRGIVDQCCTSICSLYQLENYCN

SEQ ID NO: 24 - DNA, 342 bp, synthetic construct
  source 1..342: mol_type = other DNA; note = mIns2-Hibit3 coding gene
atggccctgtggatgcgcttcctgcccctgctggccctgctcttcctctgggagtcccaccccacccaggcttttgtcaagcagcacctttgtggttcccacctggtggaggctctctacctggtgtgtggggagcgtggcttcttctacacacccatgtcccgccgtgaagtggaggacccagtgagcggctggcggctgttcaagaagattagcggtggaggcccgggagcaggtgaccttcagaccttggcactggaggtggcccagcagaagcgtggcattgtagatcagtgctgcaccagcatctgctccctctaccagctggagaactactgcaac

SEQ ID NO: 25 - protein, 114 aa, synthetic construct
  source 1..114: note = mIns2-Hibit3
MALWMRFLPLLALLFLWESHPTQAFVKQHLCGSHLVEALYLVCGERGFFYTPMSRREVEDPVSGWRLFKKISGGGPGAGDLQTLALEVAQQKRGIVDQCCTSICSLYQLENYCN

SEQ ID NO: 26 - DNA, 348 bp, synthetic construct
  source 1..348: mol_type = other DNA; note = mIns2-Hibit4 coding gene
atggccctgtggatgcgcttcctgcccctgctggccctgctcttcctctgggagtcccaccccacccaggcttttgtcaagcagcacctttgtggttcccacctggtggaggctctctacctggtgtgtggggagcgtggcttcttctacacacccatgtcccgccgtgaagtggaggacccacaagtggcacaactggagctgggtggaggcgtgagcggctggcggctgttcaagaagattagccttcagaccttggcactggaggtggcccagcagaagcgtggcattgtagatcagtgctgcaccagcatctgctccctctaccagctggagaactactgcaac

SEQ ID NO: 27 - protein, 116 aa, synthetic construct
  source 1..116: note = mIns2-Hibit4
MALWMRFLPLLALLFLWESHPTQAFVKQHLCGSHLVEALYLVCGERGFFYTPMSRREVEDPQVAQLELGGGVSGWRLFKKISLQTLALEVAQQKRGIVDQCCTSICSLYQLENYCN

SEQ ID NO: 28 - DNA, 348 bp, synthetic construct
  source 1..348: mol_type = other DNA; note = mIns2-Hibit5 coding gene
atggccctgtggatgcgcttcctgcccctgctggccctgctcttcctctgggagtcccaccccacccaggcttttgtcaagcagcacctttgtggttcccacctggtggaggctctctacctggtgtgtggggagcgtggcttcttctacacacccatgtcccgccgtgaagtggaggacccacaagtggtgagcggctggcggctgttcaagaagattagcggtggaggcccgggagcaggtgaccttcagaccttggcactggaggtggcccagcagaagcgtggcattgtagatcagtgctgcaccagcatctgctccctctaccagctggagaactactgcaac

SEQ ID NO: 29 - protein, 116 aa, synthetic construct
  source 1..116: note = mIns2-Hibit5
MALWMRFLPLLALLFLWESHPTQAFVKQHLCGSHLVEALYLVCGERGFFYTPMSRREVEDPQVVSGWRLFKKISGGGPGAGDLQTLALEVAQQKRGIVDQCCTSICSLYQLENYCN

SEQ ID NO: 30 - DNA, 373 bp, synthetic construct
  source 1..373: mol_type = other DNA; note = hIns-Hibit1 coding gene
atggccctgtggatgcgcctcctgcccctgctggcgctgctggccctctggggacctgacccagccgcagcctttgtgaaccaacacctgtgcggctcacacctggtggaagctctctacctagtgtgcggggaacgaggcttcttctacacacccaagacccgccgggaggcagaggacctgcaggtggggcaggtggagctgggcgtgagcggctggcggctgttcaagaagattagcgggggccctggtgcaggcagcctgcagcccttggccctggaggggtccctgcagaagcgtggcattgtggaacaatgctgtaccagcatctgctccctctaccagctggagaactactgcaactaagaattca

SEQ ID NO: 31 - protein, 121 aa, synthetic construct
  source 1..121: note = hIns-Hibit1
MALWMRLLPLLALLALWGPDPAAAFVNQHLCGSHLVEALYLVCGERGFFYTPKTRREAEDLQVGQVELGVSGWRLFKKISGGPGAGSLQPLALEGSLQKRGIVEQCCTSICSLYQLENYCN

SEQ ID NO: 32 - DNA, 349 bp, synthetic construct
  source 1..349: mol_type = other DNA; note = hIns-Hibit2 coding gene
atggccctgtggatgcgcctcctgcccctgctggcgctgctggccctctggggacctgacccagccgcagcctttgtgaaccaacacctgtgcggctcacacctggtggaagctctctacctagtgtgcggggaacgaggcttcttctacacacccaagacccgccgggaggcagaggacctgcaggtggggcaggtggagctgggcgggggcgtgagcggctggcggctgttcaagaagattagcttggccctggaggggtccctgcagaagcgtggcattgtggaacaatgctgtaccagcatctgctccctctaccagctggagaactactgcaactaagaattca

SEQ ID NO: 33 - protein, 113 aa, synthetic construct
  source 1..113: note = hIns-Hibit2
MALWMRLLPLLALLALWGPDPAAAFVNQHLCGSHLVEALYLVCGERGFFYTPKTRREAEDLQVGQVELGGGVSGWRLFKKISLALEGSLQKRGIVEQCCTSICSLYQLENYCN

SEQ ID NO: 34 - DNA, 358 bp, synthetic construct
  source 1..358: mol_type = other DNA; note = hIns-Hibit5 coding gene
atggccctgtggatgcgcctcctgcccctgctggcgctgctggccctctggggacctgacccagccgcagcctttgtgaaccaacacctgtgcggctcacacctggtggaagctctctacctagtgtgcggggaacgaggcttcttctacacacccaagacccgccgggaggcagaggacctgcaggtggtgagcggctggcggctgttcaagaagattagcggcgggggccctggtgcaggcagcctgcagcccttggccctggaggggtccctgcagaagcgtggcattgtggaacaatgctgtaccagcatctgctccctctaccagctggagaactactgcaactaagaattca

SEQ ID NO: 35 - protein, 116 aa, synthetic construct
  source 1..116: note = hIns-Hibit5
MALWMRLLPLLALLALWGPDPAAAFVNQHLCGSHLVEALYLVCGERGFFYTPKTRREAEDLQVVSGWRLFKKISGGGPGAGSLQPLALEGSLQKRGIVEQCCTSICSLYQLENYCN

SEQ ID NO: 36 - DNA, 3111 bp, synthetic construct
  source 1..3111: mol_type = other DNA; note = Pre-Donor-arm1-Hibit-arm2 plasmid
tctagatagcatcgtacgcgtacgtgtttggcccagatcactgtccttctgccggatccatggtgagcggctggcggctgttcaagaagattagctaagaattcaaggcctctcgagccactatagtgagtcgtattacgtagatccagacatgataagatacattgatgagtttggacaaaccacaactagaatgcagtgaaaaaaatgctttatttgtgaaatttgtgatgctattgctttatttgtaaccattataagctgcaataaacaagttaacaacaacaattgcattcattttatgtttcaggttcagggggaggtgtgggaggttttttaacgcgccgcacacaaaaaccaacacacagatcatgaaaataaagctcttttattggtaccgaattcgccagggagctctcagacgtcgcttggtcggtctttattcgaaccccagagtcccgctcacatggtttagttcctcaccttgtcgtattatactatgccgatatactatgccgatgattaattgtcaacaggctgcaggtcgaaaggcccggagatgaggaagaggagaacagcgcggcagacgtgcgcttttgaagcgtgcagaatgccgggcctccggaggaccttcgggcgcccgccccgcccctgagcccgcccctgagcccgcccccggacccaccccttcccagcctctgagcccagaaagcgaaggagcaaagctgctattggccgctgccccaaaggcctacccgcttccattgctcagcggtgctgtccatctgcacgagactagtgagacgtgctacttccatttgtcacgtcctgcacgacgcgagctgcggggcgggggggaacttcctgactaggggaggagtagaaggtggcgcgaaggggccaccaaagaacggagccggttggcgcctaccggtggatgtggaatgtgtgcgaggccagaggccacttgtgtagcgccaagtgcccagcggggctgctaaagcgcatgctccagactgccttgggaaaagcgcctcccctacccggtagaatccatggccctgtggatgcgcccaaacacgtacgcgtacgatgctcaagcttggcgctcttccgcttcctcgctcactgactcgctgcgctcggtcgttcggctgcggcgagcggtatcagctcactcaaaggcggtaatacggttatccacagaatcaggggataacgcaggaaagaacatgtgagcaaaaggccagcaaaaggccaggaaccgtaaaaaggccgcgttgctggcgtttttccataggctccgcccccctgacgagcatcacaaaaatcgacgctcaagtcagaggtggcgaaacccgacaggactataaagataccaggcgtttccccctggaagctccctcgtgcgctctcctgttccgaccctgccgcttaccggatacctgtccgcctttctcccttcgggaagcgtggcgctttctcatagctcacgctgtaggtatctcagttcggtgtaggtcgttcgctccaagctgggctgtgtgcacgaaccccccgttcagcccgaccgctgcgccttatccggtaactatcgtcttgagtccaacccggtaagacacgacttatcgccactggcagcagccactggtaacaggattagcagagcgaggtatgtaggcggtgctacagagttcttgaagtggtggcctaactacggctacactagaagaacagtatttggtatctgcgctctgctgaagccagttaccttcggaaaaagagttggtagctcttgatccggcaaacaaaccaccgctggtagcggtggtttttttgtttgcaagcagcagattacgcgcagaaaaaaaggatctcaagaagatcctttgatcttttctacggggtctgacgctcagtggaacgaaaactcacgttaagggattttggtcatgagattatcaaaaaggatcttcacctagatccttttaaattaaaaatgaagttttaaatcaatctaaagtatatatgagtaaacttggtctgacagttaccaatgcttaatcagtgaggcacctatctcagcgatctgtctatttcgttcatccatagttgcctgactccccgtcgtgtagataactacgatacgggagggcttaccatctggccccagtgctgcaatgataccgcgagatccacgctcaccggctccagatttatcagcaataaaccagccagccggaagggccgagcgcagaagtggtcctgcaactttatccgcctccatccagtctattaattgttgccgggaagctagagtaagtagttcgccagttaatagtttgcgcaacgttgttgccattgctacaggcatcgtggtgtcacgctcgtcgtttggtatggcttcattcagctccggttcccaacgatcaaggcgagttacatgatcccccatgttgtgcaaaaaagcggttagctccttcggtcctccgatcgttgtcagaagtaagttggccgcagtgttatcactcatggttatggcagcactgcataattctcttactgtcatgccatccgtaagatgcttttctgtgactggtgagtactcaaccaagtcattctgagaatagtgtatgcggcgaccgagttgctcttgcccggcgtcaatacgggataataccgcgccacatagcagaactttaaaagtgctcatcattggaaaacgttcttcggggcgaaaactctcaaggatcttaccgctgttgagatccagttcgatgtaacccactcgtgcacccaactgatcttcagcatcttttactttcaccagcgtttctgggtgagcaaaaacaggaaggcaaaatgccgcaaaaaagggaataagggcgacacggaaatgttgaatactcatactcttcctttttcaatattattgaagcatttatcagggttattgtctcatgagcggatacatatttgaatgtatttagaaaaataaacaaataggggttccgcgcacatttccccgaaaagtgccacctgacgtctaagaaaccattattatcatgacattaacctataaaaataggcgtatcacgaggccctttcgtc

SEQ ID NO: 37 - DNA, 29 bp, synthetic construct
  source 1..29: mol_type = other DNA; note = primer neoRdonorF
ccgatcccatggtttagttcctcaccttg

SEQ ID NO: 38 - DNA, 24 bp, synthetic construct
  source 1..24: mol_type = other DNA; note = primer neoRdonorR
cttctgagcgggactctggggttc

SEQ ID NO: 39 - DNA, 27 bp, synthetic construct
  source 1..27: mol_type = other DNA; note = primer inFneoRr
aaaccatgggatcggccattgaacaag

SEQ ID NO: 40 - DNA, 30 bp, synthetic construct
  source 1..30: mol_type = other DNA; note = primer inFneoRf
agtcccgctcagaagaactcgtcaagaagg

SEQ ID NO: 41 - DNA, 1902 bp, synthetic construct
  source 1..1902: mol_type = other DNA; note = Pre-Donor-arm1-NeoR-arm2
tctagatagcatcgtacgcgtacgtgtttggcccagatcactgtccttctgccggatccatggtgagcggctggcggctgttcaagaagattagctaagaattcaaggcctctcgagccactatagtgagtcgtattacgtagatccagacatgataagatacattgatgagtttggacaaaccacaactagaatgcagtgaaaaaaatgctttatttgtgaaatttgtgatgctattgctttatttgtaaccattataagctgcaataaacaagttaacaacaacaattgcattcattttatgtttcaggttcagggggaggtgtgggaggttttttaacgcgccgcacacaaaaaccaacacacagatcatgaaaataaagctcttttattggtaccgaattcgccagggagctctcagacgtcgcttggtcggtctttattcgaaccccagagtcccgctcagaagaactcgtcaagaaggcgatagaaggcgatgcgctgcgaatcgggagcggcgataccgtaaagcacgaggaagcggtcagcccattcgccgccaagctcttcagcaatatcacgggtagccaacgctatgtcctgatagcggtccgccacacccagccggccacagtcgatgaatccagaaaagcggccattttccaccatgatattcggcaagcaggcatcgccatgggtcacgacgagatcctcgccgtcgggcatgcgcgccttgagcctggcgaacagttcggctggcgcgagcccctgatgctcttcgtccagatcatcctgatcgacaagaccggcttccatccgagtacgtgctcgctcgatgcgatgtttcgcttggtggtcgaatgggcaggtagccggatcaagcgtatgcagccgccgcattgcatcagccatgatggatactttctcggcaggagcaaggtgagatgacaggagatcctgccccggcacttcgcccaatagcagccagtcccttcccgcttcagtgacaacgtcgagcacagctgcgcaaggaacgcccgtcgtggccagccacgatagccgcgctgcctcgtcctgcagttcattcagggcaccggacaggtcggtcttgacaaaaagaaccgggcgcccctgcgctgacagccggaacacggcggcatcagagcagccgattgtctgttgtgcccagtcatagccgaatagcctctccacccaagcggccggagaacctgcgtgcaatccatcttgttcaatggccgatcccatggtttagttcctcaccttgtcgtattatactatgccgatatactatgccgatgattaattgtcaacaggctgcaggtcgaaaggcccggagatgaggaagaggagaacagcgcggcagacgtgcgcttttgaagcgtgcagaatgccgggcctccggaggaccttcgggcgcccgccccgcccctgagcccgcccctgagcccgcccccggacccaccccttcccagcctctgagcccagaaagcgaaggagcaaagctgctattggccgctgccccaaaggcctacccgcttccattgctcagcggtgctgtccatctgcacgagactagtgagacgtgctacttccatttgtcacgtcctgcacgacgcgagctgcggggcgggggggaacttcctgactaggggaggagtagaaggtggcgcgaaggggccaccaaagaacggagccggttggcgcctaccggtggatgtggaatgtgtgcgaggccagaggccacttgtgtagcgccaagtgcccagcggggctgctaaagcgcatgctccagactgccttgggaaaagcgcctcccctacccggtagaatccatggccctgtggatgcgcccaaacacgtacgcgtacgatgctcaagctt

SEQ ID NO: 42 - DNA, 21 bp, synthetic construct
  source 1..21: mol_type = other DNA; note = primer DonorR
ccatggatccggcagaaggac

SEQ ID NO: 43 - DNA, 21 bp, synthetic construct
  source 1..21: mol_type = other DNA; note = primer DonorF
ctaagaattcaaggcctctcg

SEQ ID NO: 44 - DNA, 22 bp, synthetic construct
  source 1..22: mol_type = other DNA; note = primer hInsHiBitF
ctgccggatccatggccctgtg

SEQ ID NO: 45 - DNA, 21 bp, synthetic construct
  source 1..21: mol_type = other DNA; note = primer hInsHiBitR
cgagaggccttgaattcttag

SEQ ID NO: 46 - DNA, 2229 bp, synthetic construct
  source 1..2229: mol_type = other DNA; note = Arm1-hIns-Hibit1-NeoR-Arm2
tctagatagcatcgtacgcgtacgtgtttggcccagatcactgtccttctgccggatccatggccctgtggatgcgcctcctgcccctgctggcgctgctggccctctggggacctgacccagccgcagcctttgtgaaccaacacctgtgcggctcacacctggtggaagctctctacctagtgtgcggggaacgaggcttcttctacacacccaagacccgccgggaggcagaggacctgcaggtggggcaggtggagctgggcgtgagcggctggcggctgttcaagaagattagcgggggccctggtgcaggcagcctgcagcccttggccctggaggggtccctgcagaagcgtggcattgtggaacaatgctgtaccagcatctgctccctctaccagctggagaactactgcaactaagaattcaaggcctctcgagccactatagtgagtcgtattacgtagatccagacatgataagatacattgatgagtttggacaaaccacaactagaatgcagtgaaaaaaatgctttatttgtgaaatttgtgatgctattgctttatttgtaaccattataagctgcaataaacaagttaacaacaacaattgcattcattttatgtttcaggttcagggggaggtgtgggaggttttttaacgcgccgcacacaaaaaccaacacacagatcatgaaaataaagctcttttattggtaccgaattcgccagggagctctcagacgtcgcttggtcggtctttattcgaaccccagagtcccgctcagaagaactcgtcaagaaggcgatagaaggcgatgcgctgcgaatcgggagcggcgataccgtaaagcacgaggaagcggtcagcccattcgccgccaagctcttcagcaatatcacgggtagccaacgctatgtcctgatagcggtccgccacacccagccggccacagtcgatgaatccagaaaagcggccattttccaccatgatattcggcaagcaggcatcgccatgggtcacgacgagatcctcgccgtcgggcatgcgcgccttgagcctggcgaacagttcggctggcgcgagcccctgatgctcttcgtccagatcatcctgatcgacaagaccggcttccatccgagtacgtgctcgctcgatgcgatgtttcgcttggtggtcgaatgggcaggtagccggatcaagcgtatgcagccgccgcattgcatcagccatgatggatactttctcggcaggagcaaggtgagatgacaggagatcctgccccggcacttcgcccaatagcagccagtcccttcccgcttcagtgacaacgtcgagcacagctgcgcaaggaacgcccgtcgtggccagccacgatagccgcgctgcctcgtcctgcagttcattcagggcaccggacaggtcggtcttgacaaaaagaaccgggcgcccctgcgctgacagccggaacacggcggcatcagagcagccgattgtctgttgtgcccagtcatagccgaatagcctctccacccaagcggccggagaacctgcgtgcaatccatcttgttcaatggccgatcccatggtttagttcctcaccttgtcgtattatactatgccgatatactatgccgatgattaattgtcaacaggctgcaggtcgaaaggcccggagatgaggaagaggagaacagcgcggcagacgtgcgcttttgaagcgtgcagaatgccgggcctccggaggaccttcgggcgcccgccccgcccctgagcccgcccctgagcccgcccccggacccaccccttcccagcctctgagcccagaaagcgaaggagcaaagctgctattggccgctgccccaaaggcctacccgcttccattgctcagcggtgctgtccatctgcacgagactagtgagacgtgctacttccatttgtcacgtcctgcacgacgcgagctgcggggcgggggggaacttcctgactaggggaggagtagaaggtggcgcgaaggggccaccaaagaacggagccggttggcgcctaccggtggatgtggaatgtgtgcgaggccagaggccacttgtgtagcgccaagtgcccagcggggctgctaaagcgcatgctccagactgccttgggaaaagcgcctcccctacccggtagaatccatggccctgtggatgcgcccaaacacgtacgcgtacgatgctcaagctt

SEQ ID NO: 47 - DNA, 8791 bp, synthetic construct
  source 1..8791: mol_type = other DNA; note = Guide RNA-hCAS9 plasmid
gagggcctatttcccatgattccttcatatttgcatatacgatacaaggctgttagagagataattggaattaatttgactgtaaacacaaagatattagtacaaaatacgtgacgtagaaagtaataatttcttgggtagtttgcagttttaaaattatgttttaaaatggactatcatatgcttaccgtaacttgaaagtatttcgatttcttggctttatatatcttgtggaaaggacgaaacaccgagatcactgtccttctgccagttttagagctagaaatagcaagttaaaataaggctagtccgttatcaacttgaaaaagtggcaccgagtcggtgcttttttggccggccgagggcctatttcccatgattccttcatatttgcatatacgatacaaggctgttagagagataattggaattaatttgactgtaaacacaaagatattagtacaaaatacgtgacgtagaaagtaataatttcttgggtagtttgcagttttaaaattatgttttaaaatggactatcatatgcttaccgtaacttgaaagtatttcgatttcttggctttatatatcttgtggaaaggacgaaacaccggcatcgtacgcgtacgtgttgttttagagctagaaatagcaagttaaaataaggctagtccgttatcaacttgaaaaagtggcaccgagtcggtgcttttttgtctagaggtacccgttacataacttacggtaaatggcccgcctggctgaccgcccaacgacccccgcccattgacgtcaatagtaacgccaatagggactttccattgacgtcaatgggtggagtatttacggtaaactgcccacttggcagtacatcaagtgtatcatatgccaagtacgccccctattgacgtcaatgacggtaaatggcccgcctggcattgtgcccagtacatgaccttatgggactttcctacttggcagtacatctacgtattagtcatcgctattaccatggtcgaggtgagccccacgttctgcttcactctccccatctcccccccctccccacccccaattttgtatttatttattttttaattattttgtgcagcgatgggggcggggggggggggggggcgcgcgccaggcggggcggggcggggcgaggggcggggcggggcgaggcggagaggtgcggcggcagccaatcagagcggcgcgctccgaaagtttccttttatggcgaggcggcggcggcggcggccctataaaaagcgaagcgcgcggcgggcgggagtcgctgcgcgctgccttcgccccgtgccccgctccgccgccgcctcgcgccgcccgccccggctctgactgaccgcgttactcccacaggtgagcgggcgggacggcccttctcctccgggctgtaattagctgagcaagaggtaagggtttaagggatggttggttggtggggtattaatgtttaattacctggagcacctgcctgaaatcactttttttcaggttggaccggtgccaccatggactataaggaccacgacggagactacaaggatcatgatattgattacaaagacgatgacgataagatggccccaaagaagaagcggaaggtcggtatccacggagtcccagcagccgacaagaagtacagcatcggcctggacatcggcaccaactctgtgggctgggccgtgatcaccgacgagtacaaggtgcccagcaagaaattcaaggtgctgggcaacaccgaccggcacagcatcaagaagaacctgatcggagccctgctgttcgacagcggcgaaacagccgaggccacccggctgaagagaaccgccagaagaagatacaccagacggaagaaccggatctgctatctgcaagagatcttcagcaacgagatggccaaggtggacgacagcttcttccacagactggaagagtccttcctggtggaagaggataagaagcacgagcggcaccccatcttcggcaacatcgtggacgaggtggcctaccacgagaagtaccccaccatctaccacctgagaaagaaactggtggacagcaccgacaaggccgacctgcggctgatctatctggccctggcccacatgatcaagttccggggccacttcctgatcgagggcgacctgaaccccgacaacagcgacgtggacaagctgttcatccagctggtgcagacctacaaccagctgttcgaggaaaaccccatcaacgccagcggcgtggacgccaaggccatcctgtctgccagactgagcaagagcagacggctggaaaatctgatcgcccagctgcccggcgagaagaagaatggcctgttcggaaacctgattgccctgagcctgggcctgacccccaacttcaagagcaacttcgacctggccgaggatgccaaactgcagctgagcaaggacacctacgacgacgacctggacaacctgctggcccagatcggcgaccagtacgccgacctgtttctggccgccaagaacctgtccgacgccatcctgctgagcgacatcctgagagtgaacaccgagatcaccaaggcccccctgagcgcctctatgatcaagagatacgacgagcaccaccaggacctgaccctgctgaaagctctcgtgcggcagcagctgcctgagaagtacaaagagattttcttcgaccagagcaagaacggctacgccggctacattgacggcggagccagccaggaagagttctacaagttcatcaagcccatcctggaaaagatggacggcaccgaggaactgctcgtgaagctgaacagagaggacctgctgcggaagcagcggaccttcgacaacggcagcatcccccaccagatccacctgggagagctgcacgccattctgcggcggcaggaagatttttacccattcctgaaggacaaccgggaaaagatcgagaagatcctgaccttccgcatcccctactacgtgggccctctggccaggggaaacagcagattcgcctggatgaccagaaagagcgaggaaaccatcaccccctggaacttcgaggaagtggtggacaagggcgcttccgcccagagcttcatcgagcggatgaccaacttcgataagaacctgcccaacgagaaggtgctgcccaagcacagcctgctgtacgagtacttcaccgtgtataacgagctgaccaaagtgaaatacgtgaccgagggaatgagaaagcccgccttcctgagcggcgagcagaaaaaggccatcgtggacctgctgttcaagaccaaccggaaagtgaccgtgaagcagctgaaagaggactacttcaagaaaatcgagtgcttcgactccgtggaaatctccggcgtggaagatcggttcaacgcctccctgggcacataccacgatctgctgaaaattatcaaggacaaggacttcctggacaatgaggaaaacgaggacattctggaagatatcgtgctgaccctgacactgtttgaggacagagagatgatcgaggaacggctgaaaacctatgcccacctgttcgacgacaaagtgatgaagcagctgaagcggcggagatacaccggctggggcaggctgagccggaagctgatcaacggcatccgggacaagcagtccggcaagacaatcctggatttcctgaagtccgacggcttcgccaacagaaacttcatgcagctgatccacgacgacagcctgacctttaaagaggacatccagaaagcccaggtgtccggccagggcgatagcctgcacgagcacattgccaatctggccggcagccccgccattaagaagggcatcctgcagacagtgaaggtggtggacgagctcgtgaaagtgatgggccggcacaagcccgagaacatcgtgatcgaaatggccagagagaaccagaccacccagaagggacagaagaacagccgcgagagaatgaagcggatcgaagagggcatcaaagagctgggcagccagatcctgaaagaacaccccgtggaaaacacccagctgcagaacgagaagctgtacctgtactacctgcagaatgggcgggatatgtacgtggaccaggaactggacatcaaccggctgtccgactacgatgtggaccatatcgtgcctcagagctttctgaaggacgactccatcgacaacaaggtgctgaccagaagcgacaagaaccggggcaagagcgacaacgtgccctccgaagaggtcgtgaagaagatgaagaactactggcggcagctgctgaacgccaagctgattacccagagaaagttcgacaatctgaccaaggccgagagaggcggcctgagcgaactggataaggccggcttcatcaagagacagctggtggaaacccggcagatcacaaagcacgtggcacagatcctggactcccggatgaacactaagtacgacgagaatgacaagctgatccgggaagtgaaagtgatcaccctgaagtccaagctggtgtccgatttccggaaggatttccagttttacaaagtgcgcgagatcaacaactaccaccacgcccacgacgcctacctgaacgccgtcgtgggaaccgccctgatcaaaaagtaccctaagctggaaagcgagttcgtgtacggcgactacaaggtgtacgacgtgcggaagatgatcgccaagagcgagcaggaaatcggcaaggctaccgccaagtacttcttctacagcaacatcatgaactttttcaagaccgagattaccctggccaacggcgagatccggaagcggcctctgatcgagacaaacggcgaaaccggggagatcgtgtgggataagggccgggattttgccaccgtgcggaaagtgctgagcatgccccaagtgaatatcgtgaaaaagaccgaggtgcagacaggcggcttcagcaaagagtctatcctgcccaagaggaacagcgataagctgatcgccagaaagaaggactgggaccctaagaagtacggcggcttcgacagccccaccgtggcctattctgtgctggtggtggccaaagtggaaaagggcaagtccaagaaactgaagagtgtgaaagagctgctggggatcaccatcatggaaagaagcagcttcgagaagaatcccatcgactttctggaagccaagggctacaaagaagtgaaaaaggacctgatcatcaagctgcctaagtactccctgttcgagctggaaaacggccggaagagaatgctggcctctgccggcgaactgcagaagggaaacgaactggccctgccctccaaatatgtgaacttcctgtacctggccagccactatgagaagctgaagggctcccccgaggataatgagcagaaacagctgtttgtggaacagcacaagcactacctggacgagatcatcgagcagatcagcgagttctccaagagagtgatcctggccgacgctaatctggacaaagtgctgtccgcctacaacaagcaccgggataagcccatcagagagcaggccgagaatatcatccacctgtttaccctgaccaatctgggagcccctgccgccttcaagtactttgacaccaccatcgaccggaagaggtacaccagcaccaaagaggtgctggacgccaccctgatccaccagagcatcaccggcctgtacgagacacggatcgacctgtctcagctgggaggcgacaaaaggccggcggccacgaaaaaggccggccaggcaaaaaagaaaaagtaagaattcctagagctcgctgatcagcctcgactgtgccttctagttgccagccatctgttgtttgcccctcccccgtgccttccttgaccctggaaggtgccactcccactgtcctttcctaataaaatgaggaaattgcatcgcattgtctgagtaggtgtcattctattctggggggtggggtggggcaggacagcaagggggaggattgggaagagaatagcaggcatgctggggagcggccgcaggaacccctagtgatggagttggccactccctctctgcgcgctcgctcgctcactgaggccgggcgaccaaaggtcgcccgacgcccgggctttgcccgggcggcctcagtgagcgagcgagcgcgcagctgcctgcaggggcgcctgatgcggtattttctccttacgcatctgtgcggtatttcacaccgcatacgtcaaagcaaccatagtacgcgccctgtagcggcgcattaagcgcggcgggtgtggtggttacgcgcagcgtgaccgctacacttgccagcgccttagcgcccgctcctttcgctttcttcccttcctttctcgccacgttcgccggctttccccgtcaagctctaaatcgggggctccctttagggttccgatttagtgctttacggcacctcgaccccaaaaaacttgatttgggtgatggttcacgtagtgggccatcgccctgatagacggtttttcgccctttgacgttggagtccacgttctttaatagtggactcttgttccaaactggaacaacactcaactctatctcgggctattcttttgatttataagggattttgccgatttcggtctattggttaaaaaatgagctgatttaacaaaaatttaacgcgaattttaacaaaatattaacgtttacaattttatggtgcactctcagtacaatctgctctgatgccgcatagttaagccagccccgacacccgccaacacccgctgacgcgccctgacgggcttgtctgctcccggcatccgcttacagacaagctgtgaccgtctccgggagctgcatgtgtcagaggttttcaccgtcatcaccgaaacgcgcgagacgaaagggcctcgtgatacgcctatttttataggttaatgtcatgataataatggtttcttagacgtcaggtggcacttttcggggaaatgtgcgcggaacccctatttgtttatttttctaaatacattcaaatatgtatccgctcatgagacaataaccctgataaatgcttcaataatattgaaaaaggaagagtatgagtattcaacatttccgtgtcgcccttattcccttttttgcggcattttgccttcctgtttttgctcacccagaaacgctggtgaaagtaaaagatgctgaagatcagttgggtgcacgagtgggttacatcgaactggatctcaacagcggtaagatccttgagagttttcgccccgaagaacgttttccaatgatgagcacttttaaagttctgctatgtggcgcggtattatcccgtattgacgccgggcaagagcaactcggtcgccgcatacactattctcagaatgacttggttgagtactcaccagtcacagaaaagcatcttacggatggcatgacagtaagagaattatgcagtgctgccataaccatgagtgataacactgcggccaacttacttctgacaacgatcggaggaccgaaggagctaaccgcttttttgcacaacatgggggatcatgtaactcgccttgatcgttgggaaccggagctgaatgaagccataccaaacgacgagcgtgacaccacgatgcctgtagcaatggcaacaacgttgcgcaaactattaactggcgaactacttactctagcttcccggcaacaattaatagactggatggaggcggataaagttgcaggaccacttctgcgctcggcccttccggctggctggtttattgctgataaatctggagccggtgagcgtggaagccgcggtatcattgcagcactggggccagatggtaagccctcccgtatcgtagttatctacacgacggggagtcaggcaactatggatgaacgaaatagacagatcgctgagataggtgcctcactgattaagcattggtaactgtcagaccaagtttactcatatatactttagattgatttaaaacttcatttttaatttaaaaggatctaggtgaagatcctttttgataatctcatgaccaaaatcccttaacgtgagttttcgttccactgagcgtcagaccccgtagaaaagatcaaaggatcttcttgagatcctttttttctgcgcgtaatctgctgcttgcaaacaaaaaaaccaccgctaccagcggtggtttgtttgccggatcaagagctaccaactctttttccgaaggtaactggcttcagcagagcgcagataccaaatactgttcttctagtgtagccgtagttaggccaccacttcaagaactctgtagcaccgcctacatacctcgctctgctaatcctgttaccagtggctgctgccagtggcgataagtcgtgtcttaccgggttggactcaagacgatagttaccggataaggcgcagcggtcgggctgaacggggggttcgtgcacacagcccagcttggagcgaacgacctacaccgaactgagatacctacagcgtgagctatgagaaagcgccacgcttcccgaagggagaaaggcggacaggtatccggtaagcggcagggtcggaacaggagagcgcacgagggagcttccagggggaaacgcctggtatctttatagtcctgtcgggtttcgccacctctgacttgagcgtcgatttttgtgatgctcgtcaggggggcggagcctatggaaaaacgccagcaacgcggcctttttacggttcctggccttttgctggccttttgctcacatgt

SEQ ID NO: 48 - DNA, 22 bp, synthetic construct
  source 1..22: mol_type = other DNA; note = primer Ins1
gtctcccagatcactgtccttc

SEQ ID NO: 49 - DNA, 22 bp, synthetic construct
  source 1..22: mol_type = other DNA; note = primer Ins2r
tcttccccatctcctgactatg

SEQ ID NO: 50 - DNA, 22 bp, synthetic construct
  source 1..22: mol_type = other DNA; note = primer HibitR
aatcttcttgaacagccgccag

SEQ ID NO: 51 - protein, 9 aa, synthetic construct
YPYDVPDYA

SEQ ID NO: 52 - protein, 8 aa, synthetic construct
DYKDDDDK

SEQ ID NO: 53 - DNA, 44 bp, synthetic construct
  source 1..44: mol_type = other DNA
cctcactaaaggggtaccatggccctgtggatgcgcctcctgcc

SEQ ID NO: 54 - DNA, 49 bp, synthetic construct
  source 1..49: mol_type = other DNA
aagcttatcgataccgtctcactagttgcagtagttctccagctggtag

SEQ ID NO: 55 - DNA, 333 bp, synthetic construct
  source 1..333: mol_type = other DNA
atggccctgtggatgcgcctcctgcccctgctggcgctgctggccctctggggacctgacccagccgcagcctttgtgaaccaacacctgtgcggctcacacctggtggaagctctctacctagtgtgcggggaacgaggcttcttctacacacccaagacccgccgggaggcagaggacctgcaggtggggcaggtggagctgggcgggggccctggtgcaggcagcctgcagcccttggccctggaggggtccctgcagaagcgtggcattgtggaacaatgctgtaccagcatctgctccctctaccagctggagaactactgcaactag

SEQ ID NO: 56 - protein, 110 aa, synthetic construct
MALWMRLLPLLALLALWGPDPAAAFVNQHLCGSHLVEALYLVCGERGFFYTPKTRREAEDLQVGQVELGGGPGAGSLQPLALEGSLQKRGIVEQCCTSICSLYQLENYCN

SEQ ID NO: 57 - DNA, 42 bp, synthetic construct
  source 1..42: mol_type = other DNA
ctggaacatcgtatgggtacacctgcaggtcctctgcctccc

SEQ ID NO: 58 - DNA, 47 bp, synthetic construct
  source 1..47: mol_type = other DNA
ccatacgatgttccagattacgctggcgggggccctggtgcaggcag

SEQ ID NO: 59 - DNA, 345 bp, synthetic construct
  source 1..345: mol_type = other DNA
atggccctgtggatgcgcctcctgcccctgctggcgctgctggccctctggggacctgacccagccgcagcctttgtgaaccaacacctgtgcggctcacacctggtggaagctctctacctagtgtgcggggaacgaggcttcttctacacacccaagacccgccgggaggcagaggacctgcaggtgtacccatacgatgttccagattacgctggcgggggccctggtgcaggcagcctgcagcccttggccctggaggggtccctgcagaagcgtggcattgtggaacaatgctgtaccagcatctgctccctctaccagctggagaactactgcaactaa

SEQ ID NO: 60 - protein, 114 aa, synthetic construct
MALWMRLLPLLALLALWGPDPAAAFVNQHLCGSHLVEALYLVCGERGFFYTPKTRREAEDLQVYPYDVPDYAGGGPGAGSLQPLALEGSLQKRGIVEQCCTSICSLYQLENYCN

SEQ ID NO: 61 - DNA, 42 bp, synthetic construct
  source 1..42: mol_type = other DNA
cgtcgtcatccttgtaatccacctgcaggtcctctgcctccc

SEQ ID NO: 62 - DNA, 43 bp, synthetic construct
  source 1..43: mol_type = other DNA
acaaggatgacgacgataagggcgggggccctggtgcaggcag

SEQ ID NO: 63 - DNA, 349 bp, synthetic construct
  source 1..349: mol_type = other DNA
atggccctgtggatgcgcctcctgcccctgctggcgctgctggccctctggggacctgacccagccgcagcctttgtgaaccaacacctgtgcggctcacacctggtggaagctctctacctagtgtgcggggaacgaggcttcttctacacacccaagacccgccgggaggcagaggacctgcaggtggattacaaggatgacgacgataagggcgggggccctggtgcaggcagcctgcagcccttggccctggaggggtccctgcagaagcgtggcattgtggaacaatgctgtaccagcatctgctccctctaccagctggagaactactgcaactaagaattca

SEQ ID NO: 64 - protein, 113 aa, synthetic construct
MALWMRLLPLLALLALWGPDPAAAFVNQHLCGSHLVEALYLVCGERGFFYTPKTRREAEDLQVDYKDDDDKGGGPGAGSLQPLALEGSLQKRGIVEQCCTSICSLYQLENYCN

SEQ ID NO: 65 - DNA, 43 bp, synthetic construct
  source 1..43: mol_type = other DNA
cctcactaaaggggtaccatgctgatgccggtccacttcctgc

SEQ ID NO: 66 - DNA, 48 bp, synthetic construct
  source 1..48: mol_type = other DNA
aagcttatcgataccgtcctacttcttcctcccaatttgcgccatcag

SEQ ID NO: 67 - DNA, 486 bp, Homo sapiens
  source 1..486: mol_type = genomic DNA
atgctgatgccggtccacttcctgctgctcctgctgctgctcctggggggccccaggacaggcctcccccacaagttctacaaagccaagcccatcttcagctgcctcaacaccgccctgtctgaggctgagaagggccagtgggaggatgcatccctgctgagcaagaggagcttccactacctgcgcagcagagacgcctcttcgggagaggaggaggagggcaaagagaaaaagactttccccatctctggggccaggggtggagccagaggcacccggtacagatacgtgtcccaagcacagcccaggggaaagccacgccaggacacggccaagagtccccaccgcaccaagttcaccctgtccctcgacgtccccaccaacatcatgaacctcctcttcaacatcgccaaggccaagaacctgcgtgcccaggcggccgccaatgcccacctgatggcgcaaattgggaggaagaagtag

SEQ ID NO: 68 - protein, 161 aa, Homo sapiens
MLMPVHFLLLLLLLLGGPRTGLPHKFYKAKPIFSCLNTALSEAEKGQWEDASLLSKRSFHYLRSRDASSGEEEEGKEKKTFPISGARGGARGTRYRYVSQAQPRGKPRQDTAKSPHRTKFTLSLDVPTNIMNLLFNIAKAKNLRAQAAANAHLMAQIGRKK

SEQ ID NO: 69 - DNA, 46 bp, synthetic construct
  source 1..46: mol_type = other DNA
cctcactaaaggggtaccatgtccgcggccgcctacatggacttcg

SEQ ID NO: 70 - DNA, 50 bp, synthetic construct
  source 1..50: mol_type = other DNA
aagcttatcgataccgtctcacaaagcgttggccagcgcctttttcgatc

SEQ ID NO: 71 - DNA, 735 bp, Homo sapiens
  source 1..735: mol_type = genomic DNA
atgtccgcggccgcctacatggacttcgtggctgcccagtgtctggtttccatttcgaaccgcgctgcggtgccggagcatggggtcgctccggacgccgagcggctgcgactacctgagcgcgaggtgaccaaggagcacggtgacccgggggacacctggaaggattactgcacactggtcaccatcgccaagagcttgttggacctgaacaagtaccgacccatccagaccccctccgtgtgcagcgacagtctggaaagtccagatgaggatatgggatccgacagcgacgtgaccaccgaatctgggtcgagtccttcccacagcccggaggagagacaggatcctggcagcgcgcccagcccgctctccctcctccatcctggagtggctgcgaaggggaaacacgcctccgaaaagaggcacaagtgcccctacagtggctgtgggaaagtctatggaaaatcctcccatctcaaagcccattacagagtgcatacaggtgaacggccctttccctgcacgtggccagactgccttaaaaagttctcccgctcagacgagctgacccgccactaccggacccacactggggaaaagcagttccgctgtccgctgtgtgagaagcgcttcatgaggagtgaccacctcacaaagcacgcccggcggcacaccgagttccaccccagcatgatcaagcgatcgaaaaaggcgctggccaacgctttgtga

SEQ ID NO: 72 - protein, 244 aa, Homo sapiens
MSAAAYMDFVAAQCLVSISNRAAVPEHGVAPDAERLRLPEREVTKEHGDPGDTWKDYCTLVTIAKSLLDLNKYRPIQTPSVCSDSLESPDEDMGSDSDVTTESGSSPSHSPEERQDPGSAPSPLSLLHPGVAAKGKHASEKRHKCPYSGCGKVYGKSSHLKAHYRVHTGERPFPCTWPDCLKKFSRSDELTRHYRTHTGEKQFRCPLCEKRFMRSDHLTKHARRHTEFHPSMIKRSKKALANAL